European Patent Application EP 4 311 861 A1, published January 31, 2024. Title: DNA-stabilized metal cluster-based nucleic acid-sensor. Applicant: Fraunhofer-Gesellschaft zur Förderung der angewandten Forschung e.V. The sequence listing filed with the application follows.

SEQUENCE LISTING (5 sequences)

SEQ ID NO: 1 - DNA, 56 bp, Artificial sequence
  Artificial nucleotide sequence
ttcccacccaccccggcccgttaaaatcgatggtaaaggttggctcgattttaacg

SEQ ID NO: 2 - DNA, 57 bp, Artificial sequence
  Artificial nucleotide sequence
gttatggcagcactgcacttacctcccccccccccaggtaagtataattctcttact

SEQ ID NO: 3 - DNA, 58 bp, Artificial sequence
  Artificial nucleotide sequence
ttcccacccaccccggcccgttcgggaattataattaccaccaaccaattcccgaacg

SEQ ID NO: 4 - DNA, 18 bp, Artificial sequence
  Artificial nucleotide sequence
ttcccacccaccccggcc

SEQ ID NO: 5 - DNA, 25 bp, Artificial sequence
  Artificial nucleotide sequence
cttacctcccccccccccaggtaag